European Patent Specification EP 3 697 914 B9, published October 4, 2023. Title: Vectors for the treatment of Friedreich’s ataxia. Applicant: FUNDACIÓ INST D'INVESTIGACIÓ EN CIÈNCIES DE LA SALUT GERMANS TRIAS I PUJOL. The sequence listing filed with the application follows.

SEQUENCE LISTING (12 sequences)

SEQ ID NO: 1 - DNA, 518 bp, Artificial Sequence
  PGK promoter
gaattccggggttggggttgcgccttttccaaggcagccctgggtctgcgcagggacgcggctgctctgggcgtggttccgggaaacgcagcggcgccgaccctgggtctcgcacattcttcacgtccgttcgcagcgtcacccggatcttcgccgctacccttgtgggccccccggcgacgcttcctgctccgcccctaagtcgggaaggttccttgcggttcgcggcgtgccggacgtgacaaacggaagccgcacgtctcactagtaccctcgcagacggacagcgccagggagcaatggcagcgcgccgaccgcgatgggctgtggccaatagcggctgctcagcagggcgcgccgagagcagcggccgggaaggggcggtgcgggaggcggggtgtggggcggtagtgtgggccctgttcctgcccgcgcggtgttccgcattctgcaagcctccggagcgcacgtcggcagtcggctccctcgttgaccgaatcaccgacctctctccccag

SEQ ID NO: 2 - DNA, 597 bp, Artificial Sequence
  WPRE
tcgacaatcaacctctggattacaaaatttgtgaaagattgactggtattcttaactatgttgctccttttacgctatgtggatacgctgctttaatgcctttgtatcatgctattgcttcccgtatggctttcattttctcctccttgtataaatcctggttgctgtctctttatgaggagttgtggcccgttgtcaggcaacgtggcgtggtgtgcactgtgtttgctgacgcaacccccactggttggggcattgccaccacctgtcagctcctttccgggactttcgctttccccctccctattgccacggcggaactcatcgccgcctgccttgcccgctgctggacaggggctcggctgttgggcactgacaattccgtggtgttgtcggggaagctgacgtcctttccatggctgctcgcctgtgttgccacctggattctgcgcgggacgtccttctgctacgtcccttcggccctcaatccagcggaccttccttcccgcggcctgctgccggctctgcggcctcttccgcgtcttcgccttcgccctcagacgagtcggatctccctttgggccgcctccccgcctg

SEQ ID NO: 3 - DNA, 631 bp, Artificial Sequence
  frataxin
atgtggactctcgggcgccgcgcagtagccggcctcctggcgtcacccagcccggcccaggcccagaccctcacccgggtcccgcggccggcagagttggccccactctgcggccgccgtggcctgcgcaccgacatcgatgcgacctgcacgccccgccgcgcaagttcgaaccagagaggtctcaaccagatttggaatgtcaaaaagcagagtgtctatttgatgaatttgaggaaatctggaactttgggccacccaggctctctagatgagaccacctatgaaagactagcagaggaaacgctggactctttagcagagttttttgaagaccttgcagacaagccatacacgtttgaggactatgatgtctcctttgggagtggtgtcttaactgtcaaactgggtggagatctaggaacctatgtgatcaacaagcagacgccaaacaagcaaatctggctatcttctccatccagtggacctaagcgttatgactggactgggaaaaactgggtgtactcccacgacggcgtgtccctccatgagctgctggccgcagagctcactaaagccttaaaaaccaaactggacttgtcttccttggcctattccggaaaagatgctt

SEQ ID NO: 4 - DNA, 1934 bp, Artificial Sequence
  PGK frataxin and WPRE cassette
gaattccggggttggggttgcgccttttccaaggcagccctgggtctgcgcagggacgcggctgctctgggcgtggttccgggaaacgcagcggcgccgaccctgggtctcgcacattcttcacgtccgttcgcagcgtcacccggatcttcgccgctacccttgtgggccccccggcgacgcttcctgctccgcccctaagtcgggaaggttccttgcggttcgcggcgtgccggacgtgacaaacggaagccgcacgtctcactagtaccctcgcagacggacagcgccagggagcaatggcagcgcgccgaccgcgatgggctgtggccaatagcggctgctcagcagggcgcgccgagagcagcggccgggaaggggcggtgcgggaggcggggtgtggggcggtagtgtgggccctgttcctgcccgcgcggtgttccgcattctgcaagcctccggagcgcacgtcggcagtcggctccctcgttgaccgaatcaccgacctctctccccagtggctaactagagaacccactgcttactggcttatcgaaattaatacgactcactatagggagacccaagctggctagcgtttaaacttaagcttggccgccaccatgtggactctcgggcgccgcgcagtagccggcctcctggcgtcacccagcccggcccaggcccagaccctcacccgggtcccgcggccggcagagttggccccactctgcggccgccgtggcctgcgcaccgacatcgatgcgacctgcacgccccgccgcgcaagttcgaaccagagaggtctcaaccagatttggaatgtcaaaaagcagagtgtctatttgatgaatttgaggaaatctggaactttgggccacccaggctctctagatgagaccacctatgaaagactagcagaggaaacgctggactctttagcagagttttttgaagaccttgcagacaagccatacacgtttgaggactatgatgtctcctttgggagtggtgtcttaactgtcaaactgggtggagatctaggaacctatgtgatcaacaagcagacgccaaacaagcaaatctggctatcttctccatccagtggacctaagcgttatgactggactgggaaaaactgggtgtactcccacgacggcgtgtccctccatgagctgctggccgcagagctcactaaagccttaaaaaccaaactggacttgtcttccttggcctattccggaaaagatgctttgcccacctagggatcggatccccgggtaccgagctcgaattctgcagatatccagcacactttgcctttctctccacaggtgtcgacaatcaacctctggattacaaaatttgtgaaagattgactggtattcttaactatgttgctccttttacgctatgtggatacgctgctttaatgcctttgtatcatgctattgcttcccgtatggctttcattttctcctccttgtataaatcctggttgctgtctctttatgaggagttgtggcccgttgtcaggcaacgtggcgtggtgtgcactgtgtttgctgacgcaacccccactggttggggcattgccaccacctgtcagctcctttccgggactttcgctttccccctccctattgccacggcggaactcatcgccgcctgccttgcccgctgctggacaggggctcggctgttgggcactgacaattccgtggtgttgtcggggaagctgacgtcctttccatggctgctcgcctgtgttgccacctggattctgcgcgggacgtccttctgctacgtcccttcggccctcaatccagcggaccttccttcccgcggcctgctgccggctctgcggcctcttccgcgtcttcgccttcgccctcagacgagtcggatctccctttgggccgcctccccgcctg

SEQ ID NO: 5 - DNA, 2458 bp, Artificial Sequence
  ITR PGK frataxin WPRE PolyA ITR
ctggcgcgctcgctcgctcactgaggccgcccgggcaaagcccgggcgtcgggcgacctttggtcgcccggcctcagtgagcgagcgagcgcgcagagagggagtggccaactccatcactaggggttcctgaattccggggttggggttgcgccttttccaaggcagccctgggtctgcgcagggacgcggctgctctgggcgtggttccgggaaacgcagcggcgccgaccctgggtctcgcacattcttcacgtccgttcgcagcgtcacccggatcttcgccgctacccttgtgggccccccggcgacgcttcctgctccgcccctaagtcgggaaggttccttgcggttcgcggcgtgccggacgtgacaaacggaagccgcacgtctcactagtaccctcgcagacggacagcgccagggagcaatggcagcgcgccgaccgcgatgggctgtggccaatagcggctgctcagcagggcgcgccgagagcagcggccgggaaggggcggtgcgggaggcggggtgtggggcggtagtgtgggccctgttcctgcccgcgcggtgttccgcattctgcaagcctccggagcgcacgtcggcagtcggctccctcgttgaccgaatcaccgacctctctccccagtggctaactagagaacccactgcttactggcttatcgaaattaatacgactcactatagggagacccaagctggctagcgtttaaacttaagcttggccgccaccatgtggactctcgggcgccgcgcagtagccggcctcctggcgtcacccagcccggcccaggcccagaccctcacccgggtcccgcggccggcagagttggccccactctgcggccgccgtggcctgcgcaccgacatcgatgcgacctgcacgccccgccgcgcaagttcgaaccagagaggtctcaaccagatttggaatgtcaaaaagcagagtgtctatttgatgaatttgaggaaatctggaactttgggccacccaggctctctagatgagaccacctatgaaagactagcagaggaaacgctggactctttagcagagttttttgaagaccttgcagacaagccatacacgtttgaggactatgatgtctcctttgggagtggtgtcttaactgtcaaactgggtggagatctaggaacctatgtgatcaacaagcagacgccaaacaagcaaatctggctatcttctccatccagtggacctaagcgttatgactggactgggaaaaactgggtgtactcccacgacggcgtgtccctccatgagctgctggccgcagagctcactaaagccttaaaaaccaaactggacttgtcttccttggcctattccggaaaagatgctttgcccacctagggatcggatccccgggtaccgagctcgaattctgcagatatccagcacactttgcctttctctccacaggtgtcgacaatcaacctctggattacaaaatttgtgaaagattgactggtattcttaactatgttgctccttttacgctatgtggatacgctgctttaatgcctttgtatcatgctattgcttcccgtatggctttcattttctcctccttgtataaatcctggttgctgtctctttatgaggagttgtggcccgttgtcaggcaacgtggcgtggtgtgcactgtgtttgctgacgcaacccccactggttggggcattgccaccacctgtcagctcctttccgggactttcgctttccccctccctattgccacggcggaactcatcgccgcctgccttgcccgctgctggacaggggctcggctgttgggcactgacaattccgtggtgttgtcggggaagctgacgtcctttccatggctgctcgcctgtgttgccacctggattctgcgcgggacgtccttctgctacgtcccttcggccctcaatccagcggaccttccttcccgcggcctgctgccggctctgcggcctcttccgcgtcttcgccttcgccctcagacgagtcggatctccctttgggccgcctccccgcctggaattcgagctcggtacgatcagctgatcagcctcgactgtgccttctagttgccagccatctgttgtttgcccctcccccgtgccttccttgaccctggaaggtgccactcccactgtcctttcctaataaaatgaggaaattgcatcgcattgtctgagtaggtgtcattctattctggggggtggggtggggcaggacagcaagggggaggattgggaagacaatagcaggcatgctggggatgcggtgggctctatggctggcgcgctcgctcgctcactgaggccgcccgggcaaagcccgggcgtcgggcgacctttggtcgcccggcctcagtgagcgagcgagcgcgcagagagggagtggccaactccatcactaggggttcct

SEQ ID NO: 6 - DNA, 105 bp, Artificial Sequence
  Linker
tggctaactagagaacccactgcttactggcttatcgaaattaatacgactcactatagggagacccaagctggctagcgtttaaacttaagcttggccgccacc

SEQ ID NO: 7 - DNA, 27 bp, Artificial Sequence
  hFXN_Tg_FW
gaacttcaaattagttcccctttcttc

SEQ ID NO: 8 - DNA, 21 bp, Artificial Sequence
  hFXN_Tg_RV
cacagccattctttgggtttc

SEQ ID NO: 9 - DNA, 18 bp, Artificial Sequence
  IC_FW
cacgtgggctccagcatt

SEQ ID NO: 10 - DNA, 22 bp, Artificial Sequence
  IC_RV
tcaccagtcatttctgcctttg

SEQ ID NO: 11 - DNA, 29 bp, Artificial Sequence
  GAA-F
gggattggttgccagtgcttaaaagttag

SEQ ID NO: 12 - DNA, 30 bp, Artificial Sequence
  GAA-R
gatctaaggaccatcatggccacacttgcc